European Patent Application EP 4 410 830 A1, published August 7, 2024. Title: 抗体および機能性物質のコンジュゲートまたはその塩、ならびにその製造に用いられる抗体誘導体および化合物またはそれらの塩. Applicant: Ajinomoto Co., Inc. The sequence listing filed with the application follows.

SEQUENCE LISTING (1 sequence)

SEQ ID NO: 1 - protein, 17 aa, synthetic construct
RGNCAYHKGQIIWCTYH